European Patent Specification EP 3 341 112 B1, published November 8, 2023. Title: METHODS AND COMPOSITIONS FOR PROTEIN PURIFICATION AND ENZYME REACTION. Applicant: The Regents of the University of California Weiss, Gregory A. Britton, Joshua Raston, Colin L. The sequence listing filed with the application follows.

SEQUENCE LISTING (27 sequences)

SEQ ID NO: 1 - DNA, 49 bp, Artificial Sequence
  Synthetic polynucleotide
gacgacgacaagatggctaattatacagaaaaattcgcagcgtggtcag

SEQ ID NO: 2 - DNA, 72 bp, Artificial Sequence
  Synthetic polynucleotide
gaggagaagcccggttcatcacaatggacattgagaaataacttttctcaattttatcactaatgatgatga

SEQ ID NO: 3 - DNA, 66 bp, Artificial Sequence
  Synthetic polynucleotide
gacgacgacaaggtagtagtagtagtagtaatggtgagcaagggcgaggaggacaacatggccatc

SEQ ID NO: 4 - DNA, 60 bp, Artificial Sequence
  Synthetic polynucleotide
gaggagaagcccggttcacttgtacagctcgtccatgccgccggtggagtggcggccctc

SEQ ID NO: 5 - DNA, 51 bp, Artificial Sequence
  Synthetic polynucleotide
gacgacgacaagatggtgaaacaaagcactattgcactggcactcttaccg

SEQ ID NO: 6 - DNA, 54 bp, Artificial Sequence
  Synthetic polynucleotide
gaggagaagcccggttcatcagtggtggtggtggtggtgtttcagccccagggc

SEQ ID NO: 7 - DNA, 45 bp, Artificial Sequencer
  Synthetic polynucleotide
gacgacgacaagatgaaaattgggataatgagcgatacccatgac

SEQ ID NO: 8 - DNA, 45 bp, Artificial Sequence
  Synthetic polynucleotide
gaggagaagcccggttcatcataacactatctccctatactcctt

SEQ ID NO: 9 - DNA, 45 bp, Artificial Sequence
  Synthetic polynucleotide
gacgacgacaagatgccaacaattaattcgattcaaacaaccgtc

SEQ ID NO: 10 - DNA, 45 bp, Artificial Sequence
  Synthetic polynucleotide
gaggagaagcccggttcatcactaaattaacgcggccgccatcac

SEQ ID NO: 11 - protein, 15 aa, Artificial Sequence
  Synthetic polypeptide
GLNDIFEAQKIEWHE

SEQ ID NO: 12 - protein, 26 aa, Artificial Sequence
  Synthetic polypeptide
KRRWKKNFIAVSAANRFKKISSSGAL

SEQ ID NO: 13 - protein, 6 aa, Artificial Sequence
  Synthetic polypeptide
EEEEEE

SEQ ID NO: 14 - protein, 13 aa, Artificial Sequence
  Synthetic polypeptidfe
GAPVPYPDPLEPR

SEQ ID NO: 15 - protein, 8 aa, Artificial Sequence
  Synthetic polypeptide
DYKDDDDK

SEQ ID NO: 16 - protein, 9 aa, Artificial Sequence
  Synthetic polypeptide
YPYDVPDYA

SEQ ID NO: 17 - protein, 6 aa, Artificial Sequence
  Synthetic polypeptide
HHHHHH

SEQ ID NO: 18 - protein, 10 aa, Artificial Sequence
  Synthetic polypeptide
EQKLISEEDL

SEQ ID NO: 19 - protein, 15 aa, Artificial Sequence
  Synthetic polypeptide
KETAAAKFERQHMDS

SEQ ID NO: 20 - protein, 38 aa, Artificial Sequence
  Synthetic polypeptide
MDEKTTGWRGGHVVEGLAGELEQLRARLEHHPQGQREP

SEQ ID NO: 21 - protein, 13 aa, Artificial Sequence
  Synthetic polypeptide
SLAELLNAGLGGS

SEQ ID NO: 22 - protein, 8 aa, Artificial Sequence
  Synthetic polypeptide
TQDPSRVG

SEQ ID NO: 23 - protein, 8 aa, Artificial Sequence
  Synthetic polypeptide
WSHPQFEK

SEQ ID NO: 24 - protein, 6 aa, Artificial Sequence
  Synthetic polypeptide
CCPGCC

SEQ ID NO: 25 - protein, 14 aa, Artificial Sequence
  Synthetic polypeptide
GKPIPNPLLGLDST

SEQ ID NO: 26 - protein, 11 aa, Artificial Sequence
  Synthetic polypeptide
YTDIEMNRLGK

SEQ ID NO: 27 - protein, 8 aa, Artificial Sequencer
  Synthetic polypeptide
DLYDDDDK